European Patent Application EP 4 386 009 A1, published June 19, 2024. Title: BISPECIFIC FUSION POLYPEPTIDE AND APPLICATION THEREOF. Applicant: YUANPU BIOTECHNOLOGY. Application EP 22855430.9, filed August 9, 2022. The sequence listing filed with the application follows.

SEQUENCE LISTING (32 sequences)

SEQ ID NO: 1 - protein, 103 aa, synthetic construct
SDTGRPFVEMYSEIPEIIHMTEGRELVIPCRVTSPNITVTLKKFPLDTLIPDGKRIIWDSRKGFIISNATYKEIGLLTCEATVNGHLYKTNYLTHRQTNTIID

SEQ ID NO: 2 - protein, 102 aa, synthetic construct
VVLSPSHGIELSVGEKLVLNCTARTELNVGIDFNWEYPSSKHQHKKLVNRDLKTQSGSEMKKFLSTLTIDGVTRSDQGLYTCAASSGLMTKKNSTFVRVHEK

SEQ ID NO: 3 - protein, 98 aa, synthetic construct
PTLNITEESHVIDTGDSLSISCRGQHPLEWAWPGAQEAPATGDKDSEDTGVVRDCEGTDARPYCKVLLLHEVHANDTGSYVCYYKYIKARIEGTTAAS

SEQ ID NO: 4 - protein, 63 aa, synthetic construct
KDAMWVPCLVSIPGLNVTLRSQSSVLWPDGQEVVWDDRRGMLVSTPLLHDALYLQCETTWGDQ

SEQ ID NO: 5 - protein, 108 aa, synthetic construct
PFLVHITGNELYDIQLLPRKSLELLVGEKLVLNCTVWAEFNSGVTFDWDYPGKQAERGKWVPERRSQQTHTELSSILTIHNVSQHDLGSYVCKANNGIQRFRESTEVI

SEQ ID NO: 6 - protein, 98 aa, synthetic construct
PTLNITEESHVIDTGDSLSISCRGQHPLEWAWPGAQEAPATGDKDSEDTGVVRDCEGTDARPYCKVLLLHEVHAQDTGSYVCYYKYIKARIEGTTAAS

SEQ ID NO: 7 - protein, 6 aa, synthetic construct
GGGSGG

SEQ ID NO: 8 - protein, 7 aa, synthetic construct
GGGSGGG

SEQ ID NO: 9 - protein, 205 aa, synthetic construct
SDTGRPFVEMYSEIPEIIHMTEGRELVIPCRVTSPNITVTLKKFPLDTLIPDGKRIIWDSRKGFIISNATYKEIGLLTCEATVNGHLYKTNYLTHRQTNTIIDVVLSPSHGIELSVGEKLVLNCTARTELNVGIDFNWEYPSSKHQHKKLVNRDLKTQSGSEMKKFLSTLTIDGVTRSDQGLYTCAASSGLMTKKNSTFVRVHEK

SEQ ID NO: 10 - protein, 305 aa, synthetic construct
YSMTPPTLNITEESHVIDTGDSLSISCRGQHPLEWAWPGAQEAPATGDKDSEDTGVVRDCEGTDARPYCKVLLLHEVHANDTGSYVCYYKYIKARIEGTTAASSYVFVRDFEQPFINKPDTLLVNRKDAMWVPCLVSIPGLNVTLRSQSSVLWPDGQEVVWDDRRGMLVSTPLLHDALYLQCETTWGDQDFLSNPFLVHITGNELYDIQLLPRKSLELLVGEKLVLNCTVWAEFNSGVTFDWDYPGKQAERGKWVPERRSQQTHTELSSILTIHNVSQHDLGSYVCKANNGIQRFRESTEVIVHE

SEQ ID NO: 11 - protein, 305 aa, synthetic construct
YSMTPPTLNITEESHVIDTGDSLSISCRGQHPLEWAWPGAQEAPATGDKDSEDTGVVRDCEGTDARPYCKVLLLHEVHAQDTGSYVCYYKYIKARIEGTTAASSYVFVRDFEQPFINKPDTLLVNRKDAMWVPCLVSIPGLNVTLRSQSSVLWPDGQEVVWDDRRGMLVSTPLLHDALYLQCETTWGDQDFLSNPFLVHITGNELYDIQLLPRKSLELLVGEKLVLNCTVWAEFNSGVTFDWDYPGKQAERGKWVPERRSQQTHTELSSILTIHNVSQHDLGSYVCKANNGIQRFRESTEVIVHE

SEQ ID NO: 12 - protein, 226 aa, synthetic construct
DKTHTCPPCPAPELLGGPSVFLFPPKPKDTLMISRTPEVTCVVVDVSHEDPEVKFNWYVDGVEVHNAKTKPREEQYNSTYRVVSVLTVLHQDWLNGKEYKCKVSNKALPAPIEKTISKAKGQPREPQVYTLPPSRDELTKNQVSLTCLVKGFYPSDIAVEWESNGQPENNYKTTPPVLDSDGSFFLYSKLTVDKSRWQQGNVFSCSVMHEALHNHYTQKSLSLSPG

SEQ ID NO: 13 - protein, 231 aa, synthetic construct
EPKSCDKTHTCPPCPAPELLGGPSVFLFPPKPKDTLMISRTPEVTCVVVDVSHEDPEVKFNWYVDGVEVHNAKTKPREEQYNSTYRVVSVLTVLHQDWLNGKEYKCKVSNKALPAPIEKTISKAKGQPREPQVYTLPPSRDELTKNQVSLTCLVKGFYPSDIAVEWESNGQPENNYKTTPPVLDSDGSFFLYSKLTVDKSRWQQGNVFSCSVMHEALHNHYTQKSLSLSPG

SEQ ID NO: 14 - protein, 226 aa, synthetic construct
DKTHTCPPCPAPELLGGPSVFLFPPKPKDTLMISRTPEVTCVVVDVSHEDPEVKFNWYVDGVEVHNAKTKPREEQYNSTYRVVSVLTVLHQDWLNGKEYKCKVSNKALPAPIEKTISKAKGQPREPQVYTLPPSRDELTKNQVSLSCAVKGFYPSDIAVEWESNGQPENNYKTTPPVLDSDGSFFLVSKLTVDKSRWQQGNVFSCSVMHEALHNHYTQKSLSLSPG

SEQ ID NO: 15 - protein, 226 aa, synthetic construct
DKTHTCPPCPAPELLGGPSVFLFPPKPKDTLMISRTPEVTCVVVDVSHEDPEVKFNWYVDGVEVHNAKTKPREEQYNSTYRVVSVLTVLHQDWLNGKEYKCKVSNKALPAPIEKTISKAKGQPREPQVYTLPPSRDELTKNQVSLWCLVKGFYPSDIAVEWESNGQPENNYKTTPPVLDSDGSFFLYSKLTVDKSRWQQGNVFSCSVMHEALHNHYTQKSLSLSPG

SEQ ID NO: 16 - protein, 251 aa, synthetic construct
EIVMTQSPSTLSASVGDRVIITCQASEIIHSWLAWYQQKPGKAPKLLIYLASTLASGVPSRFSGSGSGAEFTLTISSLQPDDFATYYCQNVYLASTNGANFGQGTKLTVLGGGGGSGGGGSGGGGSGGGGSEVQLVESGGGLVQPGGSLRLSCTASGFSLTDYYYMTWVRQAPGKGLEWVGFIDPDDDPYYATWAKGRFTISRDNSKNTLYLQMNSLRAEDTAVYYCAGGDHNSGWGLDIWGQGTLVTVSS

SEQ ID NO: 17 - protein, 742 aa, synthetic construct
SDTGRPFVEMYSEIPEIIHMTEGRELVIPCRVTSPNITVTLKKFPLDTLIPDGKRIIWDSRKGFIISNATYKEIGLLTCEATVNGHLYKTNYLTHRQTNTIIDVVLSPSHGIELSVGEKLVLNCTARTELNVGIDFNWEYPSSKHQHKKLVNRDLKTQSGSEMKKFLSTLTIDGVTRSDQGLYTCAASSGLMTKKNSTFVRVHEKDKTHTCPPCPAPELLGGPSVFLFPPKPKDTLMISRTPEVTCVVVDVSHEDPEVKFNWYVDGVEVHNAKTKPREEQYNSTYRVVSVLTVLHQDWLNGKEYKCKVSNKALPAPIEKTISKAKGQPREPQVYTLPPSRDELTKNQVSLTCLVKGFYPSDIAVEWESNGQPENNYKTTPPVLDSDGSFFLYSKLTVDKSRWQQGNVFSCSVMHEALHNHYTQKSLSLSPGGGGSGGYSMTPPTLNITEESHVIDTGDSLSISCRGQHPLEWAWPGAQEAPATGDKDSEDTGVVRDCEGTDARPYCKVLLLHEVHAQDTGSYVCYYKYIKARIEGTTAASSYVFVRDFEQPFINKPDTLLVNRKDAMWVPCLVSIPGLNVTLRSQSSVLWPDGQEVVWDDRRGMLVSTPLLHDALYLQCETTWGDQDFLSNPFLVHITGNELYDIQLLPRKSLELLVGEKLVLNCTVWAEFNSGVTFDWDYPGKQAERGKWVPERRSQQTHTELSSILTIHNVSQHDLGSYVCKANNGIQRFRESTEVIVHE

SEQ ID NO: 18 - protein, 747 aa, synthetic construct
SDTGRPFVEMYSEIPEIIHMTEGRELVIPCRVTSPNITVTLKKFPLDTLIPDGKRIIWDSRKGFIISNATYKEIGLLTCEATVNGHLYKTNYLTHRQTNTIIDVVLSPSHGIELSVGEKLVLNCTARTELNVGIDFNWEYPSSKHQHKKLVNRDLKTQSGSEMKKFLSTLTIDGVTRSDQGLYTCAASSGLMTKKNSTFVRVHEKGGGSGGYSMTPPTLNITEESHVIDTGDSLSISCRGQHPLEWAWPGAQEAPATGDKDSEDTGVVRDCEGTDARPYCKVLLLHEVHAQDTGSYVCYYKYIKARIEGTTAASSYVFVRDFEQPFINKPDTLLVNRKDAMWVPCLVSIPGLNVTLRSQSSVLWPDGQEVVWDDRRGMLVSTPLLHDALYLQCETTWGDQDFLSNPFLVHITGNELYDIQLLPRKSLELLVGEKLVLNCTVWAEFNSGVTFDWDYPGKQAERGKWVPERRSQQTHTELSSILTIHNVSQHDLGSYVCKANNGIQRFRESTEVIVHEEPKSCDKTHTCPPCPAPELLGGPSVFLFPPKPKDTLMISRTPEVTCVVVDVSHEDPEVKFNWYVDGVEVHNAKTKPREEQYNSTYRVVSVLTVLHQDWLNGKEYKCKVSNKALPAPIEKTISKAKGQPREPQVYTLPPSRDELTKNQVSLTCLVKGFYPSDIAVEWESNGQPENNYKTTPPVLDSDGSFFLYSKLTVDKSRWQQGNVFSCSVMHEALHNHYTQKSLSLSPG

SEQ ID NO: 19 - protein, 431 aa, synthetic construct
SDTGRPFVEMYSEIPEIIHMTEGRELVIPCRVTSPNITVTLKKFPLDTLIPDGKRIIWDSRKGFIISNATYKEIGLLTCEATVNGHLYKTNYLTHRQTNTIIDVVLSPSHGIELSVGEKLVLNCTARTELNVGIDFNWEYPSSKHQHKKLVNRDLKTQSGSEMKKFLSTLTIDGVTRSDQGLYTCAASSGLMTKKNSTFVRVHEKDKTHTCPPCPAPELLGGPSVFLFPPKPKDTLMISRTPEVTCVVVDVSHEDPEVKFNWYVDGVEVHNAKTKPREEQYNSTYRVVSVLTVLHQDWLNGKEYKCKVSNKALPAPIEKTISKAKGQPREPQVYTLPPSRDELTKNQVSLSCAVKGFYPSDIAVEWESNGQPENNYKTTPPVLDSDGSFFLVSKLTVDKSRWQQGNVFSCSVMHEALHNHYTQKSLSLSPG

SEQ ID NO: 20 - protein, 531 aa, synthetic construct
YSMTPPTLNITEESHVIDTGDSLSISCRGQHPLEWAWPGAQEAPATGDKDSEDTGVVRDCEGTDARPYCKVLLLHEVHAQDTGSYVCYYKYIKARIEGTTAASSYVFVRDFEQPFINKPDTLLVNRKDAMWVPCLVSIPGLNVTLRSQSSVLWPDGQEVVWDDRRGMLVSTPLLHDALYLQCETTWGDQDFLSNPFLVHITGNELYDIQLLPRKSLELLVGEKLVLNCTVWAEFNSGVTFDWDYPGKQAERGKWVPERRSQQTHTELSSILTIHNVSQHDLGSYVCKANNGIQRFRESTEVIVHEDKTHTCPPCPAPELLGGPSVFLFPPKPKDTLMISRTPEVTCVVVDVSHEDPEVKFNWYVDGVEVHNAKTKPREEQYNSTYRVVSVLTVLHQDWLNGKEYKCKVSNKALPAPIEKTISKAKGQPREPQVYTLPPSRDELTKNQVSLWCLVKGFYPSDIAVEWESNGQPENNYKTTPPVLDSDGSFFLYSKLTVDKSRWQQGNVFSCSVMHEALHNHYTQKSLSLSPG

SEQ ID NO: 21 - protein, 794 aa, synthetic construct
YSMTPPTLNITEESHVIDTGDSLSISCRGQHPLEWAWPGAQEAPATGDKDSEDTGVVRDCEGTDARPYCKVLLLHEVHAQDTGSYVCYYKYIKARIEGTTAASSYVFVRDFEQPFINKPDTLLVNRKDAMWVPCLVSIPGLNVTLRSQSSVLWPDGQEVVWDDRRGMLVSTPLLHDALYLQCETTWGDQDFLSNPFLVHITGNELYDIQLLPRKSLELLVGEKLVLNCTVWAEFNSGVTFDWDYPGKQAERGKWVPERRSQQTHTELSSILTIHNVSQHDLGSYVCKANNGIQRFRESTEVIVHEEPKSCDKTHTCPPCPAPELLGGPSVFLFPPKPKDTLMISRTPEVTCVVVDVSHEDPEVKFNWYVDGVEVHNAKTKPREEQYNSTYRVVSVLTVLHQDWLNGKEYKCKVSNKALPAPIEKTISKAKGQPREPQVYTLPPSRDELTKNQVSLTCLVKGFYPSDIAVEWESNGQPENNYKTTPPVLDSDGSFFLYSKLTVDKSRWQQGNVFSCSVMHEALHNHYTQKSLSLSPGGGGSGGGEIVMTQSPSTLSASVGDRVIITCQASEIIHSWLAWYQQKPGKAPKLLIYLASTLASGVPSRFSGSGSGAEFTLTISSLQPDDFATYYCQNVYLASTNGANFGQGTKLTVLGGGGGSGGGGSGGGGSGGGGSEVQLVESGGGLVQPGGSLRLSCTASGFSLTDYYYMTWVRQAPGKGLEWVGFIDPDDDPYYATWAKGRFTISRDNSKNTLYLQMNSLRAEDTAVYYCAGGDHNSGWGLDIWGQGTLVTVSS

SEQ ID NO: 22 - protein, 477 aa, synthetic construct
EIVMTQSPSTLSASVGDRVIITCQASEIIHSWLAWYQQKPGKAPKLLIYLASTLASGVPSRFSGSGSGAEFTLTISSLQPDDFATYYCQNVYLASTNGANFGQGTKLTVLGGGGGSGGGGSGGGGSGGGGSEVQLVESGGGLVQPGGSLRLSCTASGFSLTDYYYMTWVRQAPGKGLEWVGFIDPDDDPYYATWAKGRFTISRDNSKNTLYLQMNSLRAEDTAVYYCAGGDHNSGWGLDIWGQGTLVTVSSDKTHTCPPCPAPELLGGPSVFLFPPKPKDTLMISRTPEVTCVVVDVSHEDPEVKFNWYVDGVEVHNAKTKPREEQYNSTYRVVSVLTVLHQDWLNGKEYKCKVSNKALPAPIEKTISKAKGQPREPQVYTLPPSRDELTKNQVSLSCAVKGFYPSDIAVEWESNGQPENNYKTTPPVLDSDGSFFLVSKLTVDKSRWQQGNVFSCSVMHEALHNHYTQKSLSLSPG

SEQ ID NO: 23 - protein, 531 aa, synthetic construct; identical to SEQ ID NO: 20

SEQ ID NO: 24 - protein, 747 aa, synthetic construct
SDTGRPFVEMYSEIPEIIHMTEGRELVIPCRVTSPNITVTLKKFPLDTLIPDGKRIIWDSRKGFIISNATYKEIGLLTCEATVNGHLYKTNYLTHRQTNTIIDVVLSPSHGIELSVGEKLVLNCTARTELNVGIDFNWEYPSSKHQHKKLVNRDLKTQSGSEMKKFLSTLTIDGVTRSDQGLYTCAASSGLMTKKNSTFVRVHEKGGGSGGYSMTPPTLNITEESHVIDTGDSLSISCRGQHPLEWAWPGAQEAPATGDKDSEDTGVVRDCEGTDARPYCKVLLLHEVHANDTGSYVCYYKYIKARIEGTTAASSYVFVRDFEQPFINKPDTLLVNRKDAMWVPCLVSIPGLNVTLRSQSSVLWPDGQEVVWDDRRGMLVSTPLLHDALYLQCETTWGDQDFLSNPFLVHITGNELYDIQLLPRKSLELLVGEKLVLNCTVWAEFNSGVTFDWDYPGKQAERGKWVPERRSQQTHTELSSILTIHNVSQHDLGSYVCKANNGIQRFRESTEVIVHEEPKSCDKTHTCPPCPAPELLGGPSVFLFPPKPKDTLMISRTPEVTCVVVDVSHEDPEVKFNWYVDGVEVHNAKTKPREEQYNSTYRVVSVLTVLHQDWLNGKEYKCKVSNKALPAPIEKTISKAKGQPREPQVYTLPPSRDELTKNQVSLTCLVKGFYPSDIAVEWESNGQPENNYKTTPPVLDSDGSFFLYSKLTVDKSRWQQGNVFSCSVMHEALHNHYTQKSLSLSPG

SEQ ID NO: 25 - DNA, 2226 bp, synthetic construct
  source 1..2226: mol_type = other DNA
tccgataccggccggcctttcgtggagatgtactccgagatccccgagatcatccacatgaccgagggcagggagctggtcattccctgccgggtgaccagccccaacatcaccgtgaccctgaagaagttccctctggataccctgatccccgatggcaagcggatcatctgggactcccggaagggcttcatcatcagcaatgctacctataaggagatcggcctgctgacctgcgaggctaccgtgaacggccacctgtacaagaccaattatctgacccacaggcagaccaataccatcatcgacgtggtgctgtccccctcccacggcatcgagctgtccgtgggcgagaagctggtgctgaattgtaccgcccggaccgagctgaatgtgggcatcgactttaattgggagtatcccagctccaagcaccagcacaagaagctggtgaatagggacctgaagacccagtccggctccgagatgaagaagttcctgagcaccctgaccatcgacggcgtgacccggagcgatcagggcctgtatacctgtgctgccagctccggcctgatgaccaagaagaatagcaccttcgtgcgggtgcacgagaaggataagacccacacctgtcctccctgtcccgctcctgagctgctgggcggaccctctgtgttcctgtttccccctaagcctaaggataccctgatgatctcccggacccccgaggtgacctgtgtggtggtggatgtgtcccacgaggaccctgaggtgaagtttaattggtatgtggatggcgtggaggtgcacaatgccaagaccaagccccgggaggagcagtataattccacctaccgggtggtgtccgtgctgaccgtgctgcaccaggactggctgaatggcaaggagtacaagtgtaaggtgagcaataaggccctgcccgctcctatcgagaagaccatctccaaggctaagggccagcctcgggagccccaggtgtacaccctgccccctagcagggatgagctgaccaagaaccaggtgtccctgacctgcctggtgaagggcttttatccctccgatatcgccgtggagtgggagtccaacggccagcctgagaacaactacaagaccaccccccccgtgctggattccgacggcagctttttcctgtactccaagctgaccgtggacaagagcaggtggcagcagggcaatgtgtttagctgctccgtgatgcacgaggctctgcacaaccactacacccagaagtccctgagcctgagccctggcggcggcggatctggaggatatagcatgacccctcccaccctgaacatcaccgaggagagccacgtgatcgacaccggcgactccctgagcatcagctgcaggggccagcaccctctggagtgggcctggcctggcgctcaggaggctccagctaccggcgacaaggatagcgaggacaccggcgtggtgcgggactgtgagggcaccgacgctcggccttattgtaaggtgctgctgctgcacgaggtgcacgcccaggacaccggctcctacgtgtgttattacaagtatatcaaggctaggatcgagggcaccaccgctgcttccagctacgtgttcgtgcgggattttgagcagcctttcatcaataagcctgacaccctgctggtgaatagaaaggatgccatgtgggtgccttgcctggtgtccatccccggcctgaacgtgaccctgaggagccagagcagcgtgctgtggcccgacggccaggaggtggtgtgggacgaccggaggggcatgctggtgtccacccctctgctgcacgatgccctgtacctgcagtgcgagaccacctggggcgaccaggattttctgagcaacccctttctggtgcacatcaccggcaacgagctgtacgacatccagctgctgcccaggaagtccctggagctgctggtgggcgagaaactggtgctgaactgcaccgtgtgggctgagttcaacagcggcgtgaccttcgactgggactaccctggcaagcaggctgagcggggcaagtgggtgcctgagaggcggtcccagcagacccacaccgagctgagctccatcctgaccatccacaacgtgtcccagcacgatctgggcagctacgtgtgcaaggctaacaacggcatccagcggttccgggagagcaccgaggtcattgtgcacgag

SEQ ID NO: 26 - DNA, 2241 bp, synthetic construct
  source 1..2241: mol_type = other DNA
tccgataccggccggccctttgtggagatgtacagcgagatccccgagatcatccacatgaccgagggcagggagctggtcattccttgtagggtgacctcccctaacatcaccgtgaccctgaagaagtttcccctggacaccctgatccctgacggcaagaggatcatctgggacagcaggaagggcttcatcatctccaacgccacctacaaggagatcggcctgctgacctgtgaggctaccgtgaacggccacctgtacaagaccaattatctgacccaccggcagaccaataccatcatcgatgtggtgctgagcccttcccacggcatcgagctgtccgtgggcgagaagctggtgctgaattgcaccgctcggaccgagctgaacgtgggcatcgactttaactgggagtacccttccagcaagcaccagcacaagaagctggtgaacagggacctgaagacccagtccggcagcgagatgaagaagttcctgagcaccctgaccatcgatggcgtgacccggagcgaccagggcctgtacacctgcgctgctagcagcggcctgatgaccaagaagaatagcaccttcgtgagggtgcacgagaagggcggcggctccggaggatactccatgacccctcccaccctgaatatcaccgaggagagccacgtgatcgataccggcgattccctgtccatctcctgtcggggccagcaccctctggagtgggcctggcctggcgctcaggaggctccagctaccggcgacaaggattccgaggataccggcgtggtgcgggattgcgagggcaccgacgccaggccatattgtaaggtgctgctgctgcacgaggtgcacgctcaggataccggcagctatgtgtgctactacaagtacatcaaggctaggatcgagggcaccaccgctgccagcagctatgtgtttgtgcgggatttcgagcagccctttatcaacaagcccgataccctgctggtgaaccggaaggatgctatgtgggtgccctgcctggtgtccatccccggcctgaacgtgaccctgaggagccagtcctccgtgctgtggcctgacggccaggaggtggtgtgggatgacaggcggggcatgctggtgagcacccctctgctgcacgatgctctgtacctgcagtgcgagaccacctggggcgaccaggatttcctgtccaacccctttctggtgcacatcaccggcaacgagctgtatgatatccagctgctgcctaggaagagcctggagctgctggtgggcgagaaactggtgctgaactgcaccgtgtgggccgagttcaattccggcgtgacctttgattgggactaccccggcaagcaggccgagcggggaaagtgggtgcctgagaggcggagccagcagacccacaccgagctgagctccatcctgaccatccacaacgtgagccagcacgacctgggcagctatgtctgcaaggccaacaacggcatccagaggttccgggagtccaccgaggtcattgtgcacgaggagcccaagagctgcgacaagacccacacctgccccccttgtcctgcccctgagctgctgggcggcccttctgtgttcctgtttccccccaagcctaaggacaccctgatgatctccaggacccctgaggtgacctgcgtggtggtggacgtgagccacgaggaccctgaggtgaagtttaattggtatgtggatggcgtggaggtgcacaacgccaagaccaagcccagggaggagcagtataatagcacctacagggtggtgtccgtgctgaccgtgctgcaccaggattggctgaatggcaaggagtataagtgcaaggtgagcaataaggctctgcccgcccccatcgagaagaccatctccaaggctaagggccagcccagggagcctcaggtgtacaccctgccccctagccgggatgagctgaccaagaatcaggtgtccctgacctgtctggtgaagggcttttacccttccgacatcgctgtggagtgggagtccaacggccagcccgagaataattataagaccaccccccctgtgctggactccgacggctccttcttcctgtacagcaagctgaccgtggacaagtccaggtggcagcagggcaacgtgttcagctgctccgtgatgcacgaggctctgcacaaccactacacccagaagtccctgtccctgtcccccggc

SEQ ID NO: 27 - DNA, 1293 bp, synthetic construct
  source 1..1293: mol_type = other DNA
tccgataccggccggcctttcgtggagatgtactccgagatccccgagatcatccacatgaccgagggcagggagctggtcattccctgccgggtgaccagccccaacatcaccgtgaccctgaagaagttccctctggataccctgatccccgatggcaagcggatcatctgggactcccggaagggcttcatcatcagcaatgctacctataaggagatcggcctgctgacctgcgaggctaccgtgaacggccacctgtacaagaccaattatctgacccacaggcagaccaataccatcatcgacgtggtgctgtccccctcccacggcatcgagctgtccgtgggcgagaagctggtgctgaattgtaccgcccggaccgagctgaatgtgggcatcgactttaattgggagtatcccagctccaagcaccagcacaagaagctggtgaatagggacctgaagacccagtccggctccgagatgaagaagttcctgagcaccctgaccatcgacggcgtgacccggagcgatcagggcctgtatacctgtgctgccagctccggcctgatgaccaagaagaatagcaccttcgtgcgggtgcacgagaaggataagacccacacctgtcctccctgtcccgctcctgagctgctgggcggaccctctgtgttcctgtttccccctaagcctaaggataccctgatgatctcccggacccccgaggtgacctgtgtggtggtggatgtgtcccacgaggaccctgaggtgaagtttaattggtatgtggatggcgtggaggtgcacaatgccaagaccaagccccgggaggagcagtataattccacctaccgggtggtgtccgtgctgaccgtgctgcaccaggactggctgaatggcaaggagtacaagtgtaaggtgagcaataaggccctgcccgctcctatcgagaagaccatctccaaggctaagggccagcctcgggagccccaggtgtacaccctgccccctagcagggatgagctgaccaagaaccaggtgtccctgtcctgcgctgtgaagggcttctacccttccgacatcgctgtggagtgggagtccaacggccagcctgagaataattataagaccacccctcccgtgctggatagcgatggctcctttttcctggtgagcaagctgaccgtggacaagtcccggtggcagcagggcaacgtgtttagctgcagcgtgatgcacgaggctctgcacaaccactatacccagaagtccctgagcctgtcccctggc

SEQ ID NO: 28 - DNA, 1593 bp, synthetic construct
  source 1..1593: mol_type = other DNA
tacagcatgaccccccccaccctgaacatcaccgaggagagccacgtgatcgacaccggcgactccctgtccatctcctgcaggggccagcaccctctggagtgggcttggcccggcgctcaggaggctccagctaccggagacaaggattccgaggataccggcgtggtgagggactgtgagggcaccgacgctaggccctactgcaaggtgctgctgctgcacgaggtgcacgctcaggacaccggctcctacgtgtgctactacaagtacatcaaggccaggatcgagggcaccaccgccgcttccagctatgtgtttgtgcgggatttcgagcagccttttatcaacaagcccgataccctgctggtgaacaggaaggatgctatgtgggtgccctgcctggtgagcatccctggcctgaatgtgaccctgcggtcccagtccagcgtgctgtggcctgacggccaggaggtggtgtgggatgataggcggggcatgctggtgtccacccctctgctgcacgatgccctgtatctgcagtgtgagaccacctggggcgatcaggacttcctgtccaatcccttcctggtgcacatcaccggcaacgagctgtacgatatccagctgctgcctcggaagagcctggagctgctggtgggcgagaagctggtgctgaattgtaccgtgtgggctgagttcaattccggcgtgacctttgattgggactaccccggcaagcaggccgagcggggaaagtgggtgcctgagaggaggtcccagcagacccacaccgagctgagctccatcctgaccatccacaacgtgagccagcacgacctgggcagctacgtgtgtaaggccaacaatggcatccagcggttccgggagtccaccgaggtcattgtgcacgaggacaagacccacacctgccctccttgtcctgctcccgagctgctgggcggcccttctgtgtttctgttcccccctaagcccaaggataccctgatgatcagcaggacccctgaggtgacctgtgtggtggtggatgtgagccacgaggaccccgaggtgaagtttaactggtatgtggatggcgtggaggtgcacaacgctaagaccaagcctagggaggagcagtataactccacctaccgggtggtgtccgtgctgaccgtgctgcaccaggactggctgaacggcaaggagtacaagtgtaaggtgagcaacaaggctctgcctgcccccatcgagaagaccatcagcaaggccaagggccagcctcgggagccccaggtttataccctgccccccagcagggacgagctgaccaagaaccaggtgagcctgtggtgcctggtgaagggcttttaccccagcgacatcgccgtggagtgggagagcaacggccagcctgagaataactacaagaccacccctcctgtgctggacagcgatggcagcttctttctgtactccaagctgaccgtggataagtccaggtggcagcagggcaacgtgttcagctgcagcgtgatgcacgaggctctgcacaatcactatacccagaagtccctgtccctgtcccctggc

SEQ ID NO: 29 - DNA, 2382 bp, synthetic construct
  source 1..2382: mol_type = other DNA
tattccatgacccctcctaccctgaacatcaccgaggagtcccacgtgatcgacaccggcgactccctgtccatctcctgtaggggccagcaccctctggagtgggcttggcccggcgctcaggaggctcctgctaccggagataaggatagcgaggacaccggcgtggtgcgggattgtgagggcaccgatgctaggccctactgtaaggtgctgctgctgcacgaggtgcacgctcaggacaccggctcctatgtgtgttactacaagtacatcaaggctcggatcgagggcaccaccgccgcttccagctatgtgtttgtgagggatttcgagcagccctttatcaataagcctgataccctgctggtgaaccggaaggatgccatgtgggtgccctgtctggtgagcatccccggcctgaatgtgaccctgaggagccagagctccgtgctgtggcccgatggccaggaggtggtgtgggacgatagacggggcatgctggtgtccacccccctgctgcacgatgctctgtatctgcagtgcgagaccacctggggcgatcaggatttcctgtccaaccctttcctggtgcacatcaccggcaacgagctgtacgatatccagctgctgccccggaagagcctggagctgctggtgggcgagaagctggtgctgaattgtaccgtgtgggccgagtttaattccggcgtgaccttcgattgggactatcctggcaagcaggctgagcggggcaagtgggtgcccgagaggagatcccagcagacccacaccgagctgtccagcatcctgaccatccacaatgtgagccagcacgatctgggcagctacgtgtgtaaggctaataacggcatccagaggttccgggagagcaccgaggtcattgtgcacgaggagcccaagagctgcgataagacccacacctgccctccttgccctgctcccgagctgctgggcggaccttccgtgttcctgttcccccccaagcccaaggacaccctgatgatcagccggacccctgaggtgacctgtgtggtggtggacgtgagccacgaggaccccgaggtgaagtttaactggtatgtggacggcgtggaggtgcacaatgccaagaccaagcctcgggaggagcagtacaatagcacctatcgggtggtgtccgtgctgaccgtgctgcaccaggattggctgaatggcaaggagtacaagtgcaaggtgagcaataaggctctgcccgctcccatcgagaagaccatcagcaaggccaagggccagcctagggagcctcaggtgtataccctgcccccctccagggatgagctgaccaagaaccaggtgtccctgacctgcctggtgaagggcttttaccctagcgacatcgctgtggagtgggagtccaacggccagcccgagaacaattacaagaccaccccccctgtgctggatagcgatggctccttcttcctgtacagcaagctgaccgtggataagtccaggtggcagcagggcaacgtgttttcctgttccgtgatgcacgaggccctgcacaatcactatacccagaagagcctgagcctgagccccggcggcggaggatctggaggaggagagatcgtgatgacccagagccctagcaccctgtccgccagcgtgggcgacagggtcattatcacctgtcaggccagcgagatcatccacagctggctggcttggtatcagcagaagcccggcaaggctcctaagctgctgatctacctggcttccaccctggctagcggcgtgcctagcaggttctccggcagcggctccggcgctgagttcaccctgaccatcagcagcctgcagcctgacgactttgctacctactattgtcagaatgtgtatctggctagcaccaacggcgctaatttcggccagggcaccaagctgaccgtcctgggcggcggaggcggatctggaggtggaggatccggcggcggcggatctggtggaggaggaagcgaggtgcagctggtggagtccggcggcggactggtgcagccaggaggaagcctgcggctgtcctgcaccgcctccggattcagcctgaccgattactattacatgacctgggtgaggcaggctcctggcaagggcctggagtgggtgggcttcatcgaccctgacgatgacccttattatgctacctgggccaagggccggttcaccatctcccgggataatagcaagaacaccctgtatctgcagatgaactccctgcgggccgaggacaccgccgtgtactattgtgctggcggcgaccacaactccggctggggactggatatctggggccagggcacactggtgaccgtgagctcc

SEQ ID NO: 30 - DNA, 1431 bp, synthetic construct
  source 1..1431: mol_type = other DNA
gagatcgtgatgacccagtcccccagcaccctgtccgcctccgtgggagatagggtcattatcacctgccaggctagcgagatcatccactcctggctggcctggtaccagcagaagcccggcaaggcccccaagctgctgatctacctggctagcaccctggctagcggcgtgccttccaggttctccggcagcggcagcggcgctgagttcaccctgaccatctccagcctgcagcctgacgactttgctacctactactgtcagaacgtgtacctggcctccaccaatggcgccaatttcggccagggcaccaagctgaccgtgctgggcggcggaggcggatctggaggaggaggatccggcggcggcggatctggtggaggaggatctgaggtgcagctggtggagtccggcggcggactggtgcagccaggaggatccctgaggctgtcctgtaccgccagcggcttctccctgaccgactattattacatgacctgggtgaggcaggctcccggcaagggcctggagtgggtgggattcatcgaccctgacgatgacccttattatgccacctgggccaagggccggtttaccatcagccgggataacagcaagaataccctgtacctgcagatgaactccctgcgggctgaggataccgccgtgtattattgtgccggcggcgatcacaatagcggctggggcctggacatctggggccagggaaccctggtgaccgtgagcagcgataagacccacacctgccctccttgccccgctcctgagctgctgggcggaccatccgtgttcctgttccctcccaagcctaaggacaccctgatgatcagccggacccctgaggtgacctgcgtggtggtggacgtgtcccacgaggaccctgaggtgaagtttaattggtatgtggacggcgtggaggtgcacaatgccaagaccaagcctcgggaggagcagtacaatagcacctaccgggtggtgagcgtgctgaccgtgctccaccaggactggctgaacggcaaggagtacaagtgcaaggtgtccaacaaggctctgcctgcccccatcgagaagaccatcagcaaggccaagggccagccccgggagccacaggtttataccctgcccccctccagggacgagctgaccaagaaccaggtgtccctgtcctgcgccgtgaagggcttttatccctccgacatcgccgtggagtgggagtccaatggccagcctgagaacaactacaagaccacccctcctgtgctggacagcgatggcagcttctttctggtgagcaagctgaccgtcgacaagagccggtggcagcagggcaatgtgttctcctgtagcgtgatgcacgaggctctgcacaaccactatacccagaagtccctgtccctgtcccctggc

SEQ ID NO: 31 - DNA, 1593 bp, synthetic construct; identical to SEQ ID NO: 28
  source 1..1593: mol_type = other DNA

SEQ ID NO: 32 - DNA, 2241 bp, synthetic construct
  source 1..2241: mol_type = other DNA
agtgatactggtcgaccatttgtggaaatgtacagcgagatccccgaaatcatccacatgacagagggcagagaactggtgattccctgcagagtgacctctcctaacatcacagtgacactgaagaagtttcctctggacaccctgatccccgacggcaagcggatcatctgggattctcggaagggcttcatcatctccaacgccacctacaaagagatcggcctgctgacctgtgaagccaccgtgaacggccacctgtataagaccaactacctgacccacagacagaccaacaccatcatcgacgtggtgttatctccttcccacggcatcgagctgtccgtgggcgaaaagctggtgctgaactgtaccgctaggaccgagctgaacgtgggcatcgacttcaactgggagtatccttccagcaagcaccagcacaagaagctggtgaatagagacctgaaaacccagtccggctctgagatgaagaaatttctgagcaccctgaccatcgacggcgtgacccggtctgaccaaggtctatacacctgtgccgcctcttccggactgatgactaaaaagaactctaccttcgtgcgggtacacgagaagggcggcggctccggaggctactccatgaccccacctaccctgaatatcaccgaagagtctcacgtgatcgacaccggcgattctcttagcatctcctgccggggccagcatcctctggaatgggcttggcctggcgctcaggaagcccctgctaccggcgacaaggactccgaggacaccggcgtcgtccgggactgcgagggcaccgacgccagaccttactgcaaagtgctcctgctgcacgaggttcatgctaacgacacaggctcctacgtgtgctactacaagtacatcaaggccagaatcgaaggcaccaccgccgcttccagctatgtgtttgtgagggatttcgagcagccctttatcaacaagcctgataccctgctggtgaaccggaaggatgccatgtgggtgccttgcctggtttccatccctggcctgaatgtgacgctgagatcccagagctccgtgctgtggcctgacggccaagaggtggtgtgggacgacagaagaggcatgctggtgagcacacccctgctgcacgacgccctgtacctgcagtgcgaaacaacctggggcgaccaggacttcctgtccaaccctttcttggtgcacatcacaggcaacgagctgtacgacatccagctgctgcctcggaagtccctggaactgctggtgggcgaaaagctggtcctgaactgcaccgtgtgggccgagttcaattctggcgtgaccttcgactgggactacccaggcaagcaggctgagagaggcaaatgggtccccgagagaagatctcagcagacccataccgagctgtcctctatcctgactatccacaacgtgtctcagcacgatctgggctcctacgtgtgcaaggccaacaacggcatccagagattccgggaatctaccgaggtcatcgtgcacgaggaacctaagtcttgtgacaagacacacacctgtcctccttgtccagctcctgagttgctcggaggccctagcgtgttcctgttccccccaaagcccaaggacaccctgatgatcagccggacccctgaggtgacctgcgtcgtggtggacgtgtctcacgaagatcctgaagtgaagttcaactggtacgtggatggcgtggaagtgcataatgctaagaccaaaccccgcgaggaacagtacaactccacctacagagtggtttccgtcctgacagtgctgcaccaagattggctgaacggcaaagagtacaagtgcaaggtgtccaacaaggctctgcctgcccccatcgagaagacaatatccaaggccaagggacagcctagagagcctcaggtgtacaccttacctccttctcgggacgagctgaccaagaaccaggtttccctgacctgcctggtgaaaggcttctaccctagcgatatcgccgtggagtgggagtccaacggacagcctgagaacaactacaagacaacgcctcctgtgctggactctgatggctccttcttcctgtactccaagctgaccgtggacaagtccagatggcagcagggcaacgtgttctcctgctctgtgatgcacgaggctctgcataaccactacacacagaagtccctgtcactgtcccccgga